European Patent Application EP 4 261 282 A1, published October 18, 2023. Title: Modified polypeptide having xylanase activity. Applicant: CJ CheilJedang Corporation. The sequence listing filed with the application follows.

SEQUENCE LISTING (80 sequences)

SEQ ID NO: 1 - protein, 227 aa, Artificial Sequence
  Op Xyn
GQRLSVGGGQNQHKGVFDGFSYEIWLDNTGGSGSMTLGKGATFKAEWSAAVNRGNFLARRGLDFGSTKKATAYEYIGLDYEASYRQTASASGNSRLCVYGWFQNRGVQGVPLVEYYIIEDWVDWVPDAQGKMVTIDGAQYKIFQMDHTGPTINGGNETFKQYFSVRQQKRTSGHITVSDHFKAWANQGWGIGNLYEVTLNAEGWQSSGVADVTKLDVYTTKQGSAPR

SEQ ID NO: 2 - DNA, 684 bp, Artificial Sequence
  Op Xyn NT
ggccagaggttgagcgtcggtggtggccagaaccagcacaagggcgtcttcgatggcttcagctacgagatctggctggataacaccggcggtagcggttccatgaccctgggtaagggagctaccttcaaggctgagtggagcgcagctgtcaaccggggtaacttcctggcccgacgcggtctggatttcggctccaccaagaaggccaccgcttacgagtacatcggcctggattacgaggcaagctacaggcagactgccagcgcaagcggtaacagccgcctctgcgtctacggctggttccagaaccggggagtgcagggcgtccccctggtcgagtactacatcatcgaggattgggtcgactgggtcccggatgcgcagggaaagatggtcaccatcgatggcgcccagtacaagatcttccagatggatcacactggcccgaccatcaacggcggtaacgagaccttcaagcagtacttcagcgtccgccagcagaagcgcactagcggccacatcaccgtcagcgatcacttcaaggcgtgggccaaccagggctggggcatcggcaacctctacgaggtcacactgaacgcagagggttggcagagcagtggtgtcgccgacgtcaccaagctggatgtctacaccaccaagcagggttcggcccctcgttag

SEQ ID NO: 3 - protein, 227 aa, Artificial Sequence
  DS1(R3C+T36C)
GQCLSVGGGQNQHKGVFDGFSYEIWLDNTGGSGSMCLGKGATFKAEWSAAVNRGNFLARRGLDFGSTKKATAYEYIGLDYEASYRQTASASGNSRLCVYGWFQNRGVQGVPLVEYYIIEDWVDWVPDAQGKMVTIDGAQYKIFQMDHTGPTINGGNETFKQYFSVRQQKRTSGHITVSDHFKAWANQGWGIGNLYEVTLNAEGWQSSGVADVTKLDVYTTKQGSAPR

SEQ ID NO: 4 - DNA, 684 bp, Artificial Sequence
  DS1(R3C+T36C) nt
ggccagtgtttgagcgtcggtggtggccagaaccagcacaagggcgtcttcgatggcttcagctacgagatctggctggataacaccggcggtagcggttccatgtgtctgggtaagggagctaccttcaaggctgagtggagcgcagctgtcaaccggggtaacttcctggcccgacgcggtctggatttcggctccaccaagaaggccaccgcttacgagtacatcggcctggattacgaggcaagctacaggcagactgccagcgcaagcggtaacagccgcctctgcgtctacggctggttccagaaccggggagtgcagggcgtccccctggtcgagtactacatcatcgaggattgggtcgactgggtcccggatgcgcagggaaagatggtcaccatcgatggcgcccagtacaagatcttccagatggatcacactggcccgaccatcaacggcggtaacgagaccttcaagcagtacttcagcgtccgccagcagaagcgcactagcggccacatcaccgtcagcgatcacttcaaggcgtgggccaaccagggctggggcatcggcaacctctacgaggtcacactgaacgcagagggttggcagagcagtggtgtcgccgacgtcaccaagctggatgtctacaccaccaagcagggttcggcccctcgttag

SEQ ID NO: 5 - protein, 227 aa, Artificial Sequence
  DS2(S5C+S34C)
GQRLCVGGGQNQHKGVFDGFSYEIWLDNTGGSGCMTLGKGATFKAEWSAAVNRGNFLARRGLDFGSTKKATAYEYIGLDYEASYRQTASASGNSRLCVYGWFQNRGVQGVPLVEYYIIEDWVDWVPDAQGKMVTIDGAQYKIFQMDHTGPTINGGNETFKQYFSVRQQKRTSGHITVSDHFKAWANQGWGIGNLYEVTLNAEGWQSSGVADVTKLDVYTTKQGSAPR

SEQ ID NO: 6 - DNA, 684 bp, Artificial Sequence
  DS2(S5C+S34C) nt
ggccagaggttgtgtgtcggtggtggccagaaccagcacaagggcgtcttcgatggcttcagctacgagatctggctggataacaccggcggtagcggttgtatgaccctgggtaagggagctaccttcaaggctgagtggagcgcagctgtcaaccggggtaacttcctggcccgacgcggtctggatttcggctccaccaagaaggccaccgcttacgagtacatcggcctggattacgaggcaagctacaggcagactgccagcgcaagcggtaacagccgcctctgcgtctacggctggttccagaaccggggagtgcagggcgtccccctggtcgagtactacatcatcgaggattgggtcgactgggtcccggatgcgcagggaaagatggtcaccatcgatggcgcccagtacaagatcttccagatggatcacactggcccgaccatcaacggcggtaacgagaccttcaagcagtacttcagcgtccgccagcagaagcgcactagcggccacatcaccgtcagcgatcacttcaaggcgtgggccaaccagggctggggcatcggcaacctctacgaggtcacactgaacgcagagggttggcagagcagtggtgtcgccgacgtcaccaagctggatgtctacaccaccaagcagggttcggcccctcgttag

SEQ ID NO: 7 - protein, 227 aa, Artificial Sequence
  DS5(F20C+A41C)
GQRLSVGGGQNQHKGVFDGCSYEIWLDNTGGSGSMTLGKGCTFKAEWSAAVNRGNFLARRGLDFGSTKKATAYEYIGLDYEASYRQTASASGNSRLCVYGWFQNRGVQGVPLVEYYIIEDWVDWVPDAQGKMVTIDGAQYKIFQMDHTGPTINGGNETFKQYFSVRQQKRTSGHITVSDHFKAWANQGWGIGNLYEVTLNAEGWQSSGVADVTKLDVYTTKQGSAPR

SEQ ID NO: 8 - DNA, 684 bp, Artificial Sequence
  DS5(F20C+A41C) nt
ggccagaggttgagcgtcggtggtggccagaaccagcacaagggcgtcttcgatggctgtagctacgagatctggctggataacaccggcggtagcggttccatgaccctgggtaagggatgtaccttcaaggctgagtggagcgcagctgtcaaccggggtaacttcctggcccgacgcggtctggatttcggctccaccaagaaggccaccgcttacgagtacatcggcctggattacgaggcaagctacaggcagactgccagcgcaagcggtaacagccgcctctgcgtctacggctggttccagaaccggggagtgcagggcgtccccctggtcgagtactacatcatcgaggattgggtcgactgggtcccggatgcgcagggaaagatggtcaccatcgatggcgcccagtacaagatcttccagatggatcacactggcccgaccatcaacggcggtaacgagaccttcaagcagtacttcagcgtccgccagcagaagcgcactagcggccacatcaccgtcagcgatcacttcaaggcgtgggccaaccagggctggggcatcggcaacctctacgaggtcacactgaacgcagagggttggcagagcagtggtgtcgccgacgtcaccaagctggatgtctacaccaccaagcagggttcggcccctcgttag

SEQ ID NO: 9 - protein, 227 aa, Artificial Sequence
  DS1 + SDM4(N52P)
GQCLSVGGGQNQHKGVFDGFSYEIWLDNTGGSGSMCLGKGATFKAEWSAAVPRGNFLARRGLDFGSTKKATAYEYIGLDYEASYRQTASASGNSRLCVYGWFQNRGVQGVPLVEYYIIEDWVDWVPDAQGKMVTIDGAQYKIFQMDHTGPTINGGNETFKQYFSVRQQKRTSGHITVSDHFKAWANQGWGIGNLYEVTLNAEGWQSSGVADVTKLDVYTTKQGSAPR

SEQ ID NO: 10 - DNA, 684 bp, Artificial Sequence
  DS1 + SDM4(N52P) nt
ggccagtgtttgagcgtcggtggtggccagaaccagcacaagggcgtcttcgatggcttcagctacgagatctggctggataacaccggcggtagcggttccatgtgtctgggtaagggagctaccttcaaggctgagtggagcgcagctgtcccccggggtaacttcctggcccgacgcggtctggatttcggctccaccaagaaggccaccgcttacgagtacatcggcctggattacgaggcaagctacaggcagactgccagcgcaagcggtaacagccgcctctgcgtctacggctggttccagaaccggggagtgcagggcgtccccctggtcgagtactacatcatcgaggattgggtcgactgggtcccggatgcgcagggaaagatggtcaccatcgatggcgcccagtacaagatcttccagatggatcacactggcccgaccatcaacggcggtaacgagaccttcaagcagtacttcagcgtccgccagcagaagcgcactagcggccacatcaccgtcagcgatcacttcaaggcgtgggccaaccagggctggggcatcggcaacctctacgaggtcacactgaacgcagagggttggcagagcagtggtgtcgccgacgtcaccaagctggatgtctacaccaccaagcagggttcggcccctcgttag

SEQ ID NO: 11 - protein, 227 aa, Artificial Sequence
  DS1 + SDM7(N28G)
GQCLSVGGGQNQHKGVFDGFSYEIWLDGTGGSGSMCLGKGATFKAEWSAAVNRGNFLARRGLDFGSTKKATAYEYIGLDYEASYRQTASASGNSRLCVYGWFQNRGVQGVPLVEYYIIEDWVDWVPDAQGKMVTIDGAQYKIFQMDHTGPTINGGNETFKQYFSVRQQKRTSGHITVSDHFKAWANQGWGIGNLYEVTLNAEGWQSSGVADVTKLDVYTTKQGSAPR

SEQ ID NO: 12 - DNA, 684 bp, Artificial Sequence
  DS1 + SDM7(N28G) nt
ggccagtgtttgagcgtcggtggtggccagaaccagcacaagggcgtcttcgatggcttcagctacgagatctggctggatggcaccggcggtagcggttccatgtgtctgggtaagggagctaccttcaaggctgagtggagcgcagctgtcaaccggggtaacttcctggcccgacgcggtctggatttcggctccaccaagaaggccaccgcttacgagtacatcggcctggattacgaggcaagctacaggcagactgccagcgcaagcggtaacagccgcctctgcgtctacggctggttccagaaccggggagtgcagggcgtccccctggtcgagtactacatcatcgaggattgggtcgactgggtcccggatgcgcagggaaagatggtcaccatcgatggcgcccagtacaagatcttccagatggatcacactggcccgaccatcaacggcggtaacgagaccttcaagcagtacttcagcgtccgccagcagaagcgcactagcggccacatcaccgtcagcgatcacttcaaggcgtgggccaaccagggctggggcatcggcaacctctacgaggtcacactgaacgcagagggttggcagagcagtggtgtcgccgacgtcaccaagctggatgtctacaccaccaagcagggttcggcccctcgttag

SEQ ID NO: 13 - protein, 227 aa, Artificial Sequence
  DS1 + SDM4+SDM7(N52P+N28G)
GQCLSVGGGQNQHKGVFDGFSYEIWLDGTGGSGSMCLGKGATFKAEWSAAVPRGNFLARRGLDFGSTKKATAYEYIGLDYEASYRQTASASGNSRLCVYGWFQNRGVQGVPLVEYYIIEDWVDWVPDAQGKMVTIDGAQYKIFQMDHTGPTINGGNETFKQYFSVRQQKRTSGHITVSDHFKAWANQGWGIGNLYEVTLNAEGWQSSGVADVTKLDVYTTKQGSAPR

SEQ ID NO: 14 - DNA, 684 bp, Artificial Sequence
  DS1 + SDM4+SDM7(N52P+N28G)
ggccagtgtttgagcgtcggtggtggccagaaccagcacaagggcgtcttcgatggcttcagctacgagatctggctggatggcaccggcggtagcggttccatgtgtctgggtaagggagctaccttcaaggctgagtggagcgcagctgtcccccggggtaacttcctggcccgacgcggtctggatttcggctccaccaagaaggccaccgcttacgagtacatcggcctggattacgaggcaagctacaggcagactgccagcgcaagcggtaacagccgcctctgcgtctacggctggttccagaaccggggagtgcagggcgtccccctggtcgagtactacatcatcgaggattgggtcgactgggtcccggatgcgcagggaaagatggtcaccatcgatggcgcccagtacaagatcttccagatggatcacactggcccgaccatcaacggcggtaacgagaccttcaagcagtacttcagcgtccgccagcagaagcgcactagcggccacatcaccgtcagcgatcacttcaaggcgtgggccaaccagggctggggcatcggcaacctctacgaggtcacactgaacgcagagggttggcagagcagtggtgtcgccgacgtcaccaagctggatgtctacaccaccaagcagggttcggcccctcgttag

SEQ ID NO: 15 - protein, 227 aa, Artificial Sequence
  DS2 + SDM4(N52P)
GQRLCVGGGQNQHKGVFDGFSYEIWLDNTGGSGCMTLGKGATFKAEWSAAVPRGNFLARRGLDFGSTKKATAYEYIGLDYEASYRQTASASGNSRLCVYGWFQNRGVQGVPLVEYYIIEDWVDWVPDAQGKMVTIDGAQYKIFQMDHTGPTINGGNETFKQYFSVRQQKRTSGHITVSDHFKAWANQGWGIGNLYEVTLNAEGWQSSGVADVTKLDVYTTKQGSAPR

SEQ ID NO: 16 - DNA, 684 bp, Artificial Sequence
  DS2 + SDM4(N52P)
ggccagaggttgtgtgtcggtggtggccagaaccagcacaagggcgtcttcgatggcttcagctacgagatctggctggataacaccggcggtagcggttgtatgaccctgggtaagggagctaccttcaaggctgagtggagcgcagctgtcccccggggtaacttcctggcccgacgcggtctggatttcggctccaccaagaaggccaccgcttacgagtacatcggcctggattacgaggcaagctacaggcagactgccagcgcaagcggtaacagccgcctctgcgtctacggctggttccagaaccggggagtgcagggcgtccccctggtcgagtactacatcatcgaggattgggtcgactgggtcccggatgcgcagggaaagatggtcaccatcgatggcgcccagtacaagatcttccagatggatcacactggcccgaccatcaacggcggtaacgagaccttcaagcagtacttcagcgtccgccagcagaagcgcactagcggccacatcaccgtcagcgatcacttcaaggcgtgggccaaccagggctggggcatcggcaacctctacgaggtcacactgaacgcagagggttggcagagcagtggtgtcgccgacgtcaccaagctggatgtctacaccaccaagcagggttcggcccctcgttag

SEQ ID NO: 17 - protein, 227 aa, Artificial Sequence
  DS2 + SDM7(N28G)
GQRLCVGGGQNQHKGVFDGFSYEIWLDGTGGSGCMTLGKGATFKAEWSAAVNRGNFLARRGLDFGSTKKATAYEYIGLDYEASYRQTASASGNSRLCVYGWFQNRGVQGVPLVEYYIIEDWVDWVPDAQGKMVTIDGAQYKIFQMDHTGPTINGGNETFKQYFSVRQQKRTSGHITVSDHFKAWANQGWGIGNLYEVTLNAEGWQSSGVADVTKLDVYTTKQGSAPR

SEQ ID NO: 18 - DNA, 684 bp, Artificial Sequence
  DS2 + SDM7(N28G) nt
ggccagaggttgtgtgtcggtggtggccagaaccagcacaagggcgtcttcgatggcttcagctacgagatctggctggatggcaccggcggtagcggttgtatgaccctgggtaagggagctaccttcaaggctgagtggagcgcagctgtcaaccggggtaacttcctggcccgacgcggtctggatttcggctccaccaagaaggccaccgcttacgagtacatcggcctggattacgaggcaagctacaggcagactgccagcgcaagcggtaacagccgcctctgcgtctacggctggttccagaaccggggagtgcagggcgtccccctggtcgagtactacatcatcgaggattgggtcgactgggtcccggatgcgcagggaaagatggtcaccatcgatggcgcccagtacaagatcttccagatggatcacactggcccgaccatcaacggcggtaacgagaccttcaagcagtacttcagcgtccgccagcagaagcgcactagcggccacatcaccgtcagcgatcacttcaaggcgtgggccaaccagggctggggcatcggcaacctctacgaggtcacactgaacgcagagggttggcagagcagtggtgtcgccgacgtcaccaagctggatgtctacaccaccaagcagggttcggcccctcgttag

SEQ ID NO: 19 - protein, 227 aa, Artificial Sequence
  DS2 + SDM4+SDM7(N52P+N28G)
GQRLCVGGGQNQHKGVFDGFSYEIWLDGTGGSGCMTLGKGATFKAEWSAAVPRGNFLARRGLDFGSTKKATAYEYIGLDYEASYRQTASASGNSRLCVYGWFQNRGVQGVPLVEYYIIEDWVDWVPDAQGKMVTIDGAQYKIFQMDHTGPTINGGNETFKQYFSVRQQKRTSGHITVSDHFKAWANQGWGIGNLYEVTLNAEGWQSSGVADVTKLDVYTTKQGSAPR

SEQ ID NO: 20 - DNA, 684 bp, Artificial Sequence
  DS2 + SDM4+SDM7(N52P+N28G) nt
ggccagaggttgtgtgtcggtggtggccagaaccagcacaagggcgtcttcgatggcttcagctacgagatctggctggatggcaccggcggtagcggttgtatgaccctgggtaagggagctaccttcaaggctgagtggagcgcagctgtcccccggggtaacttcctggcccgacgcggtctggatttcggctccaccaagaaggccaccgcttacgagtacatcggcctggattacgaggcaagctacaggcagactgccagcgcaagcggtaacagccgcctctgcgtctacggctggttccagaaccggggagtgcagggcgtccccctggtcgagtactacatcatcgaggattgggtcgactgggtcccggatgcgcagggaaagatggtcaccatcgatggcgcccagtacaagatcttccagatggatcacactggcccgaccatcaacggcggtaacgagaccttcaagcagtacttcagcgtccgccagcagaagcgcactagcggccacatcaccgtcagcgatcacttcaaggcgtgggccaaccagggctggggcatcggcaacctctacgaggtcacactgaacgcagagggttggcagagcagtggtgtcgccgacgtcaccaagctggatgtctacaccaccaagcagggttcggcccctcgttag

SEQ ID NO: 21 - protein, 227 aa, Artificial Sequence
  DS5 + SDM4(N52P)
GQRLSVGGGQNQHKGVFDGCSYEIWLDNTGGSGSMTLGKGCTFKAEWSAAVPRGNFLARRGLDFGSTKKATAYEYIGLDYEASYRQTASASGNSRLCVYGWFQNRGVQGVPLVEYYIIEDWVDWVPDAQGKMVTIDGAQYKIFQMDHTGPTINGGNETFKQYFSVRQQKRTSGHITVSDHFKAWANQGWGIGNLYEVTLNAEGWQSSGVADVTKLDVYTTKQGSAPR

SEQ ID NO: 22 - DNA, 684 bp, Artificial Sequence
  DS5 + SDM4(N52P) nt
ggccagaggttgagcgtcggtggtggccagaaccagcacaagggcgtcttcgatggctgtagctacgagatctggctggataacaccggcggtagcggttccatgaccctgggtaagggatgtaccttcaaggctgagtggagcgcagctgtcccccggggtaacttcctggcccgacgcggtctggatttcggctccaccaagaaggccaccgcttacgagtacatcggcctggattacgaggcaagctacaggcagactgccagcgcaagcggtaacagccgcctctgcgtctacggctggttccagaaccggggagtgcagggcgtccccctggtcgagtactacatcatcgaggattgggtcgactgggtcccggatgcgcagggaaagatggtcaccatcgatggcgcccagtacaagatcttccagatggatcacactggcccgaccatcaacggcggtaacgagaccttcaagcagtacttcagcgtccgccagcagaagcgcactagcggccacatcaccgtcagcgatcacttcaaggcgtgggccaaccagggctggggcatcggcaacctctacgaggtcacactgaacgcagagggttggcagagcagtggtgtcgccgacgtcaccaagctggatgtctacaccaccaagcagggttcggcccctcgttag

SEQ ID NO: 23 - protein, 227 aa, Artificial Sequence
  DS5 + SDM7(N28G)
GQRLSVGGGQNQHKGVFDGCSYEIWLDGTGGSGSMTLGKGCTFKAEWSAAVNRGNFLARRGLDFGSTKKATAYEYIGLDYEASYRQTASASGNSRLCVYGWFQNRGVQGVPLVEYYIIEDWVDWVPDAQGKMVTIDGAQYKIFQMDHTGPTINGGNETFKQYFSVRQQKRTSGHITVSDHFKAWANQGWGIGNLYEVTLNAEGWQSSGVADVTKLDVYTTKQGSAPR

SEQ ID NO: 24 - DNA, 684 bp, Artificial Sequence
  DS5 + SDM7(N28G) nt
ggccagaggttgagcgtcggtggtggccagaaccagcacaagggcgtcttcgatggctgtagctacgagatctggctggatggcaccggcggtagcggttccatgaccctgggtaagggatgtaccttcaaggctgagtggagcgcagctgtcaaccggggtaacttcctggcccgacgcggtctggatttcggctccaccaagaaggccaccgcttacgagtacatcggcctggattacgaggcaagctacaggcagactgccagcgcaagcggtaacagccgcctctgcgtctacggctggttccagaaccggggagtgcagggcgtccccctggtcgagtactacatcatcgaggattgggtcgactgggtcccggatgcgcagggaaagatggtcaccatcgatggcgcccagtacaagatcttccagatggatcacactggcccgaccatcaacggcggtaacgagaccttcaagcagtacttcagcgtccgccagcagaagcgcactagcggccacatcaccgtcagcgatcacttcaaggcgtgggccaaccagggctggggcatcggcaacctctacgaggtcacactgaacgcagagggttggcagagcagtggtgtcgccgacgtcaccaagctggatgtctacaccaccaagcagggttcggcccctcgttag

SEQ ID NO: 25 - protein, 227 aa, Artificial Sequence
  DS5 + SDM4+SDM7(N52P+N28G)
GQRLSVGGGQNQHKGVFDGCSYEIWLDGTGGSGSMTLGKGCTFKAEWSAAVPRGNFLARRGLDFGSTKKATAYEYIGLDYEASYRQTASASGNSRLCVYGWFQNRGVQGVPLVEYYIIEDWVDWVPDAQGKMVTIDGAQYKIFQMDHTGPTINGGNETFKQYFSVRQQKRTSGHITVSDHFKAWANQGWGIGNLYEVTLNAEGWQSSGVADVTKLDVYTTKQGSAPR

SEQ ID NO: 26 - DNA, 684 bp, Artificial Sequence
  DS5 + SDM4+SDM7(N52P+N28G) nt
ggccagaggttgagcgtcggtggtggccagaaccagcacaagggcgtcttcgatggctgtagctacgagatctggctggatggcaccggcggtagcggttccatgaccctgggtaagggatgtaccttcaaggctgagtggagcgcagctgtcccccggggtaacttcctggcccgacgcggtctggatttcggctccaccaagaaggccaccgcttacgagtacatcggcctggattacgaggcaagctacaggcagactgccagcgcaagcggtaacagccgcctctgcgtctacggctggttccagaaccggggagtgcagggcgtccccctggtcgagtactacatcatcgaggattgggtcgactgggtcccggatgcgcagggaaagatggtcaccatcgatggcgcccagtacaagatcttccagatggatcacactggcccgaccatcaacggcggtaacgagaccttcaagcagtacttcagcgtccgccagcagaagcgcactagcggccacatcaccgtcagcgatcacttcaaggcgtgggccaaccagggctggggcatcggcaacctctacgaggtcacactgaacgcagagggttggcagagcagtggtgtcgccgacgtcaccaagctggatgtctacaccaccaagcagggttcggcccctcgttag

SEQ ID NO: 27 - DNA, 27 bp, Artificial Sequence
  primer
tggttccagaacgatggagtgcagggc

SEQ ID NO: 28 - DNA, 19 bp, Artificial Sequence
  primer
gttctggaaccagccgtag

SEQ ID NO: 29 - DNA, 27 bp, Artificial Sequence
  primer
tggttccagaacaacggagtgcagggc

SEQ ID NO: 30 - DNA, 19 bp, Artificial Sequence
  primer
gttctggaaccagccgtag

SEQ ID NO: 31 - DNA, 26 bp, Artificial Sequence
  primer
agactgccagcgcaaacggtaacagc

SEQ ID NO: 32 - DNA, 17 bp, Artificial Sequence
  primer
tgcgctggcagtctgcc

SEQ ID NO: 33 - DNA, 24 bp, Artificial Sequence
  primer
agcgcagctgtcccccggggtaac

SEQ ID NO: 34 - DNA, 18 bp, Artificial Sequence
  primer
gacagctgcgctccactc

SEQ ID NO: 35 - DNA, 27 bp, Artificial Sequence
  primer
ctggatttcggcggtaccaagaaggcc

SEQ ID NO: 36 - DNA, 18 bp, Artificial Sequence
  primer
gccgaaatccagaccgcg

SEQ ID NO: 37 - DNA, 27 bp, Artificial Sequence
  primer
ctggatttcggcaacaccaagaaggcc

SEQ ID NO: 38 - DNA, 18 bp, Artificial Sequence
  primer
gccgaaatccagaccgcg

SEQ ID NO: 39 - DNA, 23 bp, Artificial Sequence
  primer
atctggctggatggcaccggcgg

SEQ ID NO: 40 - DNA, 16 bp, Artificial Sequence
  primer
atccagccagatctcg

SEQ ID NO: 41 - DNA, 18 bp, Artificial Sequence
  primer
accgtcatcgatcacttc

SEQ ID NO: 42 - DNA, 18 bp, Artificial Sequence
  primer
gtgatcgatgacggtgat

SEQ ID NO: 43 - DNA, 21 bp, Artificial Sequence
  primer
aagcagtggttcagcgtccgc

SEQ ID NO: 44 - DNA, 24 bp, Artificial Sequence
  primer
gctgaaccactgcttgaaggtctc

SEQ ID NO: 45 - DNA, 26 bp, Artificial Sequence
  primer
agactgccagcgcannkggtaacagc

SEQ ID NO: 46 - DNA, 17 bp, Artificial Sequence
  primer
tgcgctggcagtctgcc

SEQ ID NO: 47 - DNA, 24 bp, Artificial Sequence
  primer
agcgcagctgtcnnkcggggtaac

SEQ ID NO: 48 - DNA, 18 bp, Artificial Sequence
  primer
gacagctgcgctccactc

SEQ ID NO: 49 - DNA, 26 bp, Artificial Sequence
  primer
atctggctggatnnkaccggcggtag

SEQ ID NO: 50 - DNA, 16 bp, Artificial Sequence
  primer
atccagccagatctcg

SEQ ID NO: 51 - DNA, 25 bp, Artificial Sequence
  primer
ttgagcgtcggtnnkggccagaacc

SEQ ID NO: 52 - DNA, 18 bp, Artificial Sequence
  primer
accgacgctcaacctctg

SEQ ID NO: 53 - DNA, 20 bp, Artificial Sequence
  primer
ggccagtgtttgagcgtcgg

SEQ ID NO: 54 - DNA, 22 bp, Artificial Sequence
  primer
gctcaaacactggcccatatgg

SEQ ID NO: 55 - DNA, 24 bp, Artificial Sequence
  primer
aagggatgtaccttcaaggctgag

SEQ ID NO: 56 - DNA, 24 bp, Artificial Sequence
  primer
acccagacacatggaaccgctacc

SEQ ID NO: 57 - DNA, 20 bp, Artificial Sequence
  primer
aggttgtgtgtcggtggtgg

SEQ ID NO: 58 - DNA, 21 bp, Artificial Sequence
  primer
accgacacacaacctctggcc

SEQ ID NO: 59 - DNA, 24 bp, Artificial Sequence
  primer
agcggttgtatgaccctgggtaag

SEQ ID NO: 60 - DNA, 21 bp, Artificial Sequence
  primer
ggtcatacaaccgctaccgcc

SEQ ID NO: 61 - DNA, 26 bp, Artificial Sequence
  primer
ccggattgtcagggaaagatggtcac

SEQ ID NO: 62 - DNA, 22 bp, Artificial Sequence
  primer
tccctgacaatccgggacccag

SEQ ID NO: 63 - DNA, 26 bp, Artificial Sequence
  primer
aagatctgtcagatggatcacactgg

SEQ ID NO: 64 - DNA, 25 bp, Artificial Sequence
  primer
catctgacagatcttgtactgggcg

SEQ ID NO: 65 - DNA, 21 bp, Artificial Sequence
  primer
ttcggctgtaccaagaaggcc

SEQ ID NO: 66 - DNA, 24 bp, Artificial Sequence
  primer
cttggtacagccgaaatccagacc

SEQ ID NO: 67 - DNA, 24 bp, Artificial Sequence
  primer
atcggctgtctctacgaggtcgca

SEQ ID NO: 68 - DNA, 20 bp, Artificial Sequence
  primer
gtagagacagccgatgcccc

SEQ ID NO: 69 - DNA, 24 bp, Artificial Sequence
  primer
gatggctgtagctacgagatctgg

SEQ ID NO: 70 - DNA, 23 bp, Artificial Sequence
  primer
gtagctacagccatcgaagacgc

SEQ ID NO: 71 - DNA, 24 bp, Artificial Sequence
  primer
aagggatgtaccttcaaggctgag

SEQ ID NO: 72 - DNA, 23 bp, Artificial Sequence
  primer
gaaggtacatcccttacccaggg

SEQ ID NO: 73 - DNA, 25 bp, Artificial Sequence
  primer
aaggcctgtgcttacgagtacatcg

SEQ ID NO: 74 - DNA, 23 bp, Artificial Sequence
  primer
gtaagcacaggccttcttggtgg

SEQ ID NO: 75 - DNA, 22 bp, Artificial Sequence
  primer
tggggctgtggcaacctctacg

SEQ ID NO: 76 - DNA, 19 bp, Artificial Sequence
  primer
gttgccacagccccagccc

SEQ ID NO: 77 - DNA, 23 bp, Artificial Sequence
  primer
cgcggttgtgatttcggctccac

SEQ ID NO: 78 - DNA, 21 bp, Artificial Sequence
  primer
gaaatcacaaccgcgtcgggc

SEQ ID NO: 79 - DNA, 25 bp, Artificial Sequence
  primer
ctggattgttacaccaccaagcagg

SEQ ID NO: 80 - DNA, 25 bp, Artificial Sequence
  primer
ggtgtaacaatccagcttggtgacg